European Patent Application EP 4 477 227 A1, published December 18, 2024. Title: 락토바실러스 플란타룸 균주 및 항암제를 포함하는 병용 요법을 이용한 암 예방 또는 치료용 조성물. Applicant: 지아이바이옴. The sequence listing filed with the application follows.

SEQUENCE LISTING (1 sequence)

SEQ ID NO: 1 - DNA, 1424 bp, synthetic construct
  source 1..1424: mol_type = other DNA
tcgaacgaactctggtattgattggtgcttgcatcatgatttacatttgagtgagtggcgaactggtgagtaacacgtgggaaacctgcccagaagcgggggataacacctggaaacagatgctaataccgcataacaacttggaccgcatggtccgagcttgaaagatggcttcggctatcacttttggatggtcccgcggcgtattagctagatggtggggtaacggctcaccatggcaatgatacgtagccgacctgagagggtaatcggccacattgggactgagacacggcccaaactcctacgggaggcagcagtagggaatcttccacaatggacgaaagtctgatggagcaacgccgcgtgagtgaagaagggtttcggctcgtaaaactctgttgttaaagaagaacatatctgagagtaactgttcaggtattgacggtatttaaccagaaagccacggctaactacgtgccagcagccgcggtaatacgtaggtggcaagcgttgtccggatttattgggcgtaaagcgagcgcaggcggttttttaagtctgatgtgaaagccttcggctcaaccgaagaagtgcatcggaaactgggaaacttgagtgcagaagaggacagtggaactccatgtgtagcggtgaaatgcgtagatatatggaagaacaccagtggcgaaggcggctgtctggtctgtaactgacgctgaggctcgaaagtatgggtagcaaacaggattagataccctggtagtccataccgtaaacgatgaatgctaagtgttggagggtttccgcccttcagtgctgcagctaacgcattaagcattccgcctggggagtacggccgcaaggctgaaactcaaaggaattgacgggggcccgcacaagcggtggagcatgtggtttaattcgaagctacgcgaagaaccttaccaggtcttgacatactatgcaaatctaagagattagacgttcccttcggggacatggatacaggtggtgcatggttgtcgtcagctcgtgtcgtgagatgttgggttaagtcccgcaacgagcgcaacccttattatcagttgccagcattaagttgggcactctggtgagactgccggtgacaaaccggaggaaggtggggatgacgtcaaatcatcatgccccttatgacctgggctacacacgtgctacaatggatggtacaacgagttgcgaactcgcgagagtaagctaatctcttaaagccattctcagttcggattgtaggctgcaactcgcctacatgaagtcggaatcgctagtaatcgcggatcagcatgccgcggtgaatacgttcccgggccttgtacacaccgcccgtcacaccatgagagtttgtaacacccaaagtcggtggggtaaccttttaggaacca